European Patent Specification EP 3 763 822 B1, published February 12, 2025. Title: METHOD FOR SCREENING ENDOGENOUS SKIN AGEING TARGET, ACTIVE SUBSTANCEs FOR IMPROVING ENDOGENOUS SKIN AGEING AND METHOD FOR SCREENING ACTIVE SUBSTANCES. Applicant: JALA Group COMPANY. The sequence listing filed with the application follows.

SEQUENCE LISTING (10 sequences)

SEQ ID NO: 1 - RNA, 22 nt, Homo sapiens
cugggagaaggcuguuuacucu

SEQ ID NO: 2 - RNA, 22 nt, Homo sapiens
acggguuaggcucuugggagcu

SEQ ID NO: 3 - DNA, 20 bp, Homo sapiens
aacacactgcaggagggact

SEQ ID NO: 4 - DNA, 20 bp, Homo sapiens
gctgcgtgatatttgaaagg

SEQ ID NO: 5 - DNA, 20 bp, Homo sapiens
ggttgaggtgagaggtttgc

SEQ ID NO: 6 - DNA, 20 bp, Homo sapiens
attatttgcggtgcatccat

SEQ ID NO: 7 - DNA, 20 bp, Homo sapiens
aacacactgcaggagggact

SEQ ID NO: 8 - DNA, 20 bp, Homo sapiens
tcttgctgggatcattaggg

SEQ ID NO: 9 - DNA, 22 bp, Homo sapiens
tctgtgatgcccttagatgtcc

SEQ ID NO: 10 - DNA, 20 bp, Homo sapiens
aatggggttcaacgggttac